European Patent Application EP 4 534 558 A1, published April 9, 2025. Title: ANTI-CD228 ANTIBODY AND DRGU CONJUGATE THEREOF. Applicant: SHANDONG BOAN BIOTECHNOLOGY CO., LTD. Application WO PCT/CN2023/096155, filed May 23, 2023. The sequence listing filed with the application follows.

SEQUENCE LISTING (49 sequences)

SEQ ID NO: 1 - protein, 107 aa, synthetic construct
DIQMTQSPSAMSASVGDRVTITCRASQGINNYLAWFQQKPGKVPKRLIYAASSLQSGVPSRFSGSGSGTEFTLTISSLQPEDFATYYCLQHNSYPFTFGPGTKVDIK

SEQ ID NO: 2 - protein, 124 aa, synthetic construct
EVQLVESGGGVVQPGRSLRLSCAASGFTFSSYAMHWVRQAPGKGLEWVAVISYDGSNKYYADSVKGRFTISRDNSKNTLYLQMNSLRAEDTAVYYCARGPYLAAAGTALTFDIWGQGTMVTVSS

SEQ ID NO: 3 - protein, 107 aa, synthetic construct
DIVMTQSPSSLSASVGDRVTITCRASQGISNYLAWFQQKPGKVPKLLIYAASTLQSGVPSRFSGSGSGTDFTLTISSLQPEDVATYYCQKYNSAPFTFGPGTKVDIK

SEQ ID NO: 4 - protein, 126 aa, synthetic construct
EVQLVESGGGVVQPGRSLRLSCAASGFTFSSYAMHWVRQAPGKGLEWVAVISYDGSNKYYADSVKGRFTISRDNSKNTLFLQMNSLRAEDTAVYYCARDVYHYGSRSPYYYGMDVWGQGTTVTVSS

SEQ ID NO: 5 - protein, 107 aa, synthetic construct
DIQMTQSPSSLSASVGDRVTITCRASQAISNYLAWYQQKPGKVPKLLIYAASTLHPGVPSRFSGSGSGTDFTLTISSLQPEDVATYYCQKYNSAPFTFGPGTKVDIK

SEQ ID NO: 6 - protein, 126 aa, synthetic construct
EVQLVESGGGVVQPGRSLRLSCAASGFTFSSYAMHWVRQAPGKGLEWVAVISYDGSNKYYADSVKGRFTISRDNSKNTLYLQMNSLRAEDTAVYYCARDVYHYGSRSPYYYGMDVWGQGTTVTVSS

SEQ ID NO: 7 - protein, 108 aa, synthetic construct
EIVLTQSPATLSVSPGERATLSCRASQSVSSNLAWYQQKPGQAPRHLIDGASSRASGIPDRFSGSGSGTDFTLTISRLEPEDFAVYYCQQYGSSPPFTFGPGTKVDIK

SEQ ID NO: 8 - protein, 122 aa, synthetic construct
EVQLVESGGGVVQPGRSLRLSCAASGFTFSSYAMHWVRQAPGKGLEWVAVISFDGSNKYYTDSVKGRFTISRDNSKNTLYLQMNSLRAEDTAVYYCAREVPYYYGSGPFDYWGQGTLVTVSS

SEQ ID NO: 9 - protein, 107 aa, synthetic construct
EIVLTQSPGTLSLSPGERATLSCRASQSVSSSSLAWYQQKPGQAPRHLIDGASSRASGIPDRFSGSGSGTDFTLTISRLEPEDFAVYYCQQYGSSYTFGQGTKVDIK

SEQ ID NO: 10 - protein, 122 aa, synthetic construct
EVQLVESGGGVVQPGRSLRLSCAASGFTFSSYAMHWVRQAPGKGLEWVAVISYDGSNKYYADSVKGRFTISRDNSKNTLYLQMNSLRAEDTAVYYCAREVPYYYGSGPFDYWGQGTLVTVSS

SEQ ID NO: 11 - protein, 107 aa, synthetic construct
DIQMTQSPSSVSASVGDRVTITCRASQGISSWLAWYQQKPGKAPKLLIYAASSLQSGVPSRFSGSGSGTDFTLTISSLQPEDVATYYCQKYNSAPFTFGPGTKVDIK

SEQ ID NO: 12 - protein, 126 aa, synthetic construct
EVQLVESGGGVVQPGRSLRLSCAASGFTFSSYAMHWVRQAPGKGLEWVAVISYDGSNKYHADSVKGRFTISRDNSKNTLFLQMNSLRAEDTAVYYCVRDVYHYGSRSPYYYGMDVWGQGTTVTVSS

SEQ ID NO: 13 - protein, 6 aa, synthetic construct
QGINNY

SEQ ID NO: 14 - protein, 4 aa, synthetic construct
AASS

SEQ ID NO: 15 - protein, 9 aa, synthetic construct
LQHNSYPFT

SEQ ID NO: 16 - protein, 8 aa, synthetic construct
GFTFSSYA

SEQ ID NO: 17 - protein, 8 aa, synthetic construct
ISYDGSNK

SEQ ID NO: 18 - protein, 17 aa, synthetic construct
ARGPYLAAAGTALTFDI

SEQ ID NO: 19 - protein, 6 aa, synthetic construct
QGISNY

SEQ ID NO: 20 - protein, 4 aa, synthetic construct
AAST

SEQ ID NO: 21 - protein, 10 aa, synthetic construct
QKYNSAPFTF

SEQ ID NO: 22 - protein, 19 aa, synthetic construct
ARDVYHYGSRSPYYYGMDV

SEQ ID NO: 23 - protein, 6 aa, synthetic construct
QAISNY

SEQ ID NO: 24 - protein, 6 aa, synthetic construct
QSVSSN

SEQ ID NO: 25 - protein, 4 aa, synthetic construct
GASS

SEQ ID NO: 26 - protein, 11 aa, synthetic construct
QQYGSSPPFTF

SEQ ID NO: 27 - protein, 8 aa, synthetic construct
ISFDGSNK

SEQ ID NO: 28 - protein, 15 aa, synthetic construct
AREVPYYYGSGPFDY

SEQ ID NO: 29 - protein, 7 aa, synthetic construct
QSVSSSS

SEQ ID NO: 30 - protein, 9 aa, synthetic construct
QQYGSSYTF

SEQ ID NO: 31 - protein, 6 aa, synthetic construct
QGISSW

SEQ ID NO: 32 - protein, 19 aa, synthetic construct
VRDVYHYGSRSPYYYGMDV

SEQ ID NO: 33 - protein, 330 aa, synthetic construct [sequence omitted]

SEQ ID NO: 34 - protein, 107 aa, synthetic construct [sequence omitted]

SEQ ID NO: 35 - protein, 448 aa, synthetic construct
QVQLQESGPGLVKPSETLSLTCTVSGDSITSGYWNWIRQPPGKGLEYIGYISDSGITYYNPSLKSRVTISRDTSKNQYSLKLSSVTAADTAVYYCARRTLATYYAMDYWGQGTLVTVSSASTKGPSVFPLAPSSKSTSGGTAALGCLVKDYFPEPVTVSWNSGALTSGVHTFPAVLQSSGLYSLSSVVTVPSSSLGTQTYICNVNHKPSNTKVDKKVEPKSCDKTHTCPPCPAPELLGGPSVFLFPPKPKDTLMISRTPEVTCVVVDVSHEDPEVKFNWYVDGVEVHNAKTKPREEQYNSTYRVVSVLTVLHQDWLNGKEYKCKVSNKALPAPIEKTISKAKGQPREPQVYTLPPSRDELTKNQVSLTCLVKGFYPSDIAVEWESNGQPENNYKTTPPVLDSDGSFFLYSKLTVDKSRWQQGNVFSCSVMHEALHNHYTQKSLSLSPG

SEQ ID NO: 36 - protein, 219 aa, synthetic construct
DFVMTQSPLSLPVTLGQPASISCRASQSLVHSDGNTYLHWYQQRPGQSPRLLIYRVSNRFSGVPDRFSGSGSGTDFTLKISRVEAEDVGVYYCSQSTHVPPTFGQGTKLEIKRTVAAPSVFIFPPSDEQLKSGTASVVCLLNNFYPREAKVQWKVDNALQSGNSQESVTEQDSKDSTYSLSSTLTLSKADYEKHKVYACEVTHQGLSSPVTKSFNRGEC

SEQ ID NO: 37 - protein, 456 aa, synthetic construct
EVQLVESGGGVVQPGRSLRLSCAASGFTFSSYAMHWVRQAPGKGLEWVAVISYDGSNKYYADSVKGRFTISRDNSKNTLFLQMNSLRAEDTAVYYCARDVYHYGSRSPYYYGMDVWGQGTTVTVSSASTKGPSVFPLAPSSKSTSGGTAALGCLVKDYFPEPVTVSWNSGALTSGVHTFPAVLQSSGLYSLSSVVTVPSSSLGTQTYICNVNHKPSNTKVDKKVEPKSCDKTHTCPPCPAPELLGGPSVFLFPPKPKDTLMISRTPEVTCVVVDVSHEDPEVKFNWYVDGVEVHNAKTKPREEQYNSTYRVVSVLTVLHQDWLNGKEYKCKVSNKALPAPIEKTISKAKGQPREPQVYTLPPSRDELTKNQVSLTCLVKGFYPSDIAVEWESNGQPENNYKTTPPVLDSDGSFFLYSKLTVDKSRWQQGNVFSCSVMHEALHNHYTQKSLSLSPGK

SEQ ID NO: 38 - protein, 214 aa, synthetic construct
DIQMTQSPSSLSASVGDRVTITCRASQGISNYLAWYQQKPGKVPELLIYAASTLLSGVPSRFGGSGSGTDFTLTISSLQPEDIATYYCQKYNSAPFTFGPGTKVDIKRTVAAPSVFIFPPSDEQLKSGTASVVCLLNNFYPREAKVQWKVDNALQSGNSQESVTEQDSKDSTYSLSSTLTLSKADYEKHKVYACEVTHQGLSSPVTKSFNRGEC

SEQ ID NO: 39 - protein, 452 aa, synthetic construct
EVQLVESGGGVVQPGRSLRLSCAASGFTFSSYAMHWVRQAPGKGLEWVAVISYDGSNKYYADSVKGRFTISRDNSKNTLYLQMNSLRAEDTAVYYCAREVPYYYGSGPFDYWGQGTLVTVSSASTKGPSVFPLAPSSKSTSGGTAALGCLVKDYFPEPVTVSWNSGALTSGVHTFPAVLQSSGLYSLSSVVTVPSSSLGTQTYICNVNHKPSNTKVDKKVEPKSCDKTHTCPPCPAPELLGGPSVFLFPPKPKDTLMISRTPEVTCVVVDVSHEDPEVKFNWYVDGVEVHNAKTKPREEQYNSTYRVVSVLTVLHQDWLNGKEYKCKVSNKALPAPIEKTISKAKGQPREPQVYTLPPSRDELTKNQVSLTCLVKGFYPSDIAVEWESNGQPENNYKTTPPVLDSDGSFFLYSKLTVDKSRWQQGNVFSCSVMHEALHNHYTQKSLSLSPGK

SEQ ID NO: 40 - protein, 214 aa, synthetic construct
DIQLTQSPSTLSASVGDRVTITCRASQSVSSSYLAWYQQKPGQAPRRLIDGASSRATGIPDRFSGSGSGTDFTLTISRLEPEDFAVYYCQHYGSSYTFGQGTKVEIKRTVAAPSVFIFPPSDEQLKSGTASVVCLLNNFYPREAKVQWKVDNALQSGNSQESVTEQDSKDSTYSLSSTLTLSKADYEKHKVYACEVTHQGLSSPVTKSFNRGEC

SEQ ID NO: 41 - protein, 718 aa, synthetic construct
MRGPSGALWLLLALRTVLGGMEVRWCATSDPEQHKCGNMSEAFREAGIQPSLLCVRGTSADHCVQLIAAQEADAITLDGGAIYEAGKEHGLKPVVGEVYDQEVGTSYYAVAVVRRSSHVTIDTLKGVKSCHTGINRTVGWNVPVGYLVESGRLSVMGCDVLKAVSDYFGGSCVPGAGETSYSESLCRLCRGDSSGEGVCDKSPLERYYDYSGAFRCLAEGAGDVAFVKHSTVLENTDGKTLPSWGQALLSQDFELLCRDGSRADVTEWRQCHLARVPAHAVVVRADTDGGLIFRLLNEGQRLFSHEGSSFQMFSSEAYGQKDLLFKDSTSELVPIATQTYEAWLGHEYLHAMKGLLCDPNRLPPYLRWCVLSTPEIQKCGDMAVAFRRQRLKPEIQCVSAKSPQHCMERIQAEQVDAVTLSGEDIYTAGKTYGLVPAAGEHYAPEDSSNSYYVVAVVRRDSSHAFTLDELRGKRSCHAGFGSPAGWDVPVGALIQRGFIRPKDCDVLTAVSEFFNASCVPVNNPKNYPSSLCALCVGDEQGRNKCVGNSQERYYGYRGAFRCLVENAGDVAFVRHTTVFDNTNGHNSEPWAAELRSEDYELLCPNGARAEVSQFAACNLAQIPPHAVMVRPDTNIFTVYGLLDKAQDLFGDDHNKNGFKMFDSSNYHGQDLLFKDATVRAVPVGEKTTYRGWLGLDYVAALEGMSSQQHHHHHHHHHH

SEQ ID NO: 42 - protein, 723 aa, synthetic construct
SRAATMRLLSVTFWLLLSLRTVLCVMEMQWCTISDPEQQKCKDMSKAFQGAGIQPSLLCVQGTSTDHCVQLIKDQKADAITLDGGAIYQAGKEYGLKPVVGEVYDQDIGTSYYAVAVVRRNSNVTINTLKGVKSCHTGINRTVGWNVPVGYLVETGHLSVMGCDVLKAVGDYFGGSCVPGAGETSHSESLCRLCRGDSSGHNVCDKSPLERYYDYSGAFRCLAEGAGDVAFVKHSTVLENTDGKTLPSWGKALMSQDFQLLCRDGSRADITEWRRCHLAKVPAHAVVVRDDMDGGLIFRLLNEGQLLFSHEDSSFQMFSSKAYGQKNLLFKDSTLELVPIATQNYESWLGQEYLHAMKGLLCDPNRLPHYLRWCVLSVPEIQKCGDMAVAFSRQSLKPEIQCVSAESPEHCMQQIQAGHIDAVTLRGEDIYRAGKAYGLVPAAGELYAEEDRSNSYFVVAVVRRDSSYSFTLDELRSKRSCHPGLGSPAGWEVPIGSLIQRGFIRPKDCDVLTAVSEFFNASCVPVNNPKNYPSSLCALCVGDEKGRNKCVGSSQERYYGYSGAFRCLVENAGDVAFLKHTTVFENTNGHNPEPWASHLRWQDYELLCPNGARAEVDQFQACNLAQMPSHAVMVHPDTNIFTVYGLLDKAQDLFGDDHNKNGFQMFDSSKYHSQDLLFKDATVRAVPVREKTTYLDWLGPDYVVALEGMLSQQHHHHHHHHHH

SEQ ID NO: 43 - protein, 718 aa, synthetic construct
MRGPSRALWLLLALRTVLGGMEVRWCVTSDPEQHKCSNMSTAFREAGIQPSLLCVQGTSPDHCIQLIAAQEADAITLDGGAIYEAGKEHGLKPVVGEVYDQEVGTSYYAVAVVKRSSQVTINTLKGVKSCHTGINRTVGWNVPVGYLVESGRLSVMGCDVLKAVSDYFGGSCVPGAGETRYSESLCRLCRGDSSGEGVCDKSPLERYYDYSGAFRCLVEGAGDVAFVKHSTVLENTDGKTLPSWGQALLSQDFELLCRDGSRADVTEWRQCHLARVPAHAVVVRADTDGGLIFRLLNEGQRLFSHEGSSFQMFSSEAYGQKDLLFKDSTSELVPIATQTYEAWLGQEYLHAMKGLLCDPNRLPPYLRWCVLSTPEIQKCGDMAVAFGRQQLKPEIQCVSAKSPQHCMEQIQAGQIDTVTLSGEDIYTAGKTYGLAPAAGEGYASEDSSNSYFVVAVVRRDSSHAFTLDELWGKRSCHAGFGSPAGWDIPVGALIRRGFIRPKDCDVLTAVSEFFNASCVPVNNPKNYPSSLCALCVGDEQGRNKCVGNSQERYYGNSGAFRCLVENAGDVAFVRHTTVFDNTNGHNSEPWAAELRSEDYELLCPNGARAEVSQFAACNLAQMPPHAVMVRPDTNIFTVYGLLDKAQDLFGDDHNKNGFKMFDSSNYHGQDLLFKDATVRAVPVGEKTTYRDWLGLDYVAALEGMLSQQHHHHHHHHHH

SEQ ID NO: 44 - skipped

SEQ ID NO: 45 - protein, 9 aa, synthetic construct
QKYNSAPFT

SEQ ID NO: 46 - protein, 7 aa, synthetic construct
QSVSSSY

SEQ ID NO: 47 - skipped

SEQ ID NO: 48 - protein, 8 aa, synthetic construct
QHYGSSYT

SEQ ID NO: 49 - protein, 19 aa, synthetic construct
ARDVYHYGSRSPYYYGMDV